European Patent Specification EP 3 589 115 B1, published November 12, 2025. Title: SEPTORIA RESISTANCE IN CELERY. Applicant: Bejo Zaden B.V. The sequence listing filed with the application follows.

SEQUENCE LISTING (26 sequences)

SEQ ID NO: 1 - DNA, 51 bp, Apium graveolens
cgaacccgaaacctaaagctcaacaaccaccagtgccaatgccaccatcac

SEQ ID NO: 2 - DNA, 51 bp, Apium graveolens
cgaacccgaaacctaaagctcaacaaacaccagtgccaatgccaccatcac

SEQ ID NO: 3 - DNA, 51 bp, Apium graveolens
cttcctttcagttgagctggatacaatagcatctggattaaccacaccaac

SEQ ID NO: 4 - DNA, 51 bp, Apium graveolens
cttcctttcagttgagctggatacaagagcatctggattaaccacaccaac

SEQ ID NO: 5 - DNA, 51 bp, Apium graveolens
taaaaaaagaaaaagaagaggaacaacaacacacaattctatcattaaact

SEQ ID NO: 6 - DNA, 51 bp, Apium graveolens
taaaaaaagaaaaagaagaggaacaataacacacaattctatcattaaact

SEQ ID NO: 7 - DNA, 51 bp, Apium graveolens
aatgatcaatcgtaggttgtattgcttgaacatgcccttacatgcatagaa

SEQ ID NO: 8 - DNA, 51 bp, Apium graveolens
aatgatcaatcgtaggttgtattgctcgaacatgcccttacatgcatagaa

SEQ ID NO: 9 - DNA, 51 bp, Apium graveolens
cgaacctcctctaaactctctccgcctatcccaacaaccccaacaaactcc

SEQ ID NO: 10 - DNA, 51 bp, Apium graveolens
cgaacctcctctaaactctctccgccaatcccaacaaccccaacaaactcc

SEQ ID NO: 11 - DNA, 51 bp, Apium graveolens
gctgtagcactgatactacaccatcaggctcttgatakagagagttctttg

SEQ ID NO: 12 - DNA, 51 bp, Apium graveolens
gctgtagcactgatactacaccatcatgctcttgatakagagagttctttg

SEQ ID NO: 13 - DNA, 51 bp, Apium graveolens
tccattcttccacttctcaacaatgccggatcaagtttctctacatgatta

SEQ ID NO: 14 - DNA, 51 bp, Apium graveolens
tccattcttccacttctcaacaatgcaggatcaagtttctctacatgatta

SEQ ID NO: 15 - DNA, 51 bp, Apium graveolens
gatattgggtcagggtgagaacaagctagcccaaccagtaacactctcctc

SEQ ID NO: 16 - DNA, 51 bp, Apium graveolens
gatattgggtcagggtgagaacaagccagcccaaccagtaacactctcctc

SEQ ID NO: 17 - DNA, 51 bp, Apium graveolens
agttctagcctgctacttgctactctgctactcagaagcagaggcgtccga

SEQ ID NO: 18 - DNA, 51 bp, Apium graveolens
agttctagcctgctacttgctactctcctactcagaagcagaggcgtccga

SEQ ID NO: 19 - DNA, 51 bp, Apium graveolens
gatttttgagctaaaagaattgctgtttgtttgagatgttacatacaaaaa

SEQ ID NO: 20 - DNA, 51 bp, Apium graveolens
gatttttgagctaaaagaattgctgtctgtttgagatgttacatacaaaaa

SEQ ID NO: 21 - DNA, 51 bp, Apium graveolens
tgcatccattagcaacgacaaccctgcgctagtttcatgtgttgatgatga

SEQ ID NO: 22 - DNA, 51 bp, Apium graveolens
tgcatccattagcaacgacaaccctgtgctagtttcatgtgttgatgatga

SEQ ID NO: 23 - DNA, 51 bp, Apium graveolens
atttctccatacagatggcattcttttgagttgatamtatacagtgcagcc

SEQ ID NO: 24 - DNA, 51 bp, Apium graveolens
atttctccatacagatggcattctttcgagttgatamtatacagtgcagcc

SEQ ID NO: 25 - DNA, 51 bp, Apium graveolens
aaaggttatcgtcaagtacttcaaatgtttcctctcttgacaaaaagatya

SEQ ID NO: 26 - DNA, 51 bp, Apium graveolens
aaaggttatcgtcaagtacttcaaatctttcctctcttgacaaaaagatya